European Patent Application EP 4 170 026 A1, published April 26, 2023. Title: MICROBIAL PRODUCTION OF ALKANOLAMIDES AND AMIDOAMINES AND USES THEREOF. Applicant: Genomatica, Inc. Application EP. The sequence listing filed with the application follows.

SEQUENCE LISTING (22 sequences)

SEQ ID NO: 1 - protein, 207 aa, unidentified
  source 1..207: note = Uncultured bacterium
MESLYNGDGFVIARATALEEIEESVTLFEAVSAEMGWSPGDRLRAYAANAEYLMALVGGALAGAVQIVLSNGHDPMPSDHVWPELAAGRRYDLAHASVMALAPRFRGAAGLFGPLGVEMWRLCRDAGKSEIWIECVPRNLAVYRRCGWPLEVAGELRTHFGEPCYLARMGVEAVAESLRARAGRCDGFARLVAQAYRDTGWRSMGLA

SEQ ID NO: 2 - DNA, 624 bp, unidentified
  source 1..624: mol_type = genomic DNA; note = Uncultured bacterium
atggaaagtttgtacaatggcgacggattcgtcatcgcaagggcgacggccctggaagagatcgaggagtcggtcacactcttcgaggcggtctccgccgaaatgggatggagccctggggatcggcttcgggcatacgcagcgaacgcggagtacctgatggcgctagtcggcggagcgctggctggggcggtgcagatcgtgctctccaacggtcacgatcctatgccttcggaccacgtctggccggaacttgcggcgggtcgacgatatgaccttgcgcacgcgtcagtgatggcgcttgccccgcgcttccggggagcggcaggactattcgggccgcttggcgtcgagatgtggaggctttgccgggacgccgggaaatccgagatatggatcgagtgcgtgccgaggaaccttgcggtgtaccgaagatgtggttggccgctggaggtggcgggcgagttgcggacccatttcggcgagccttgctacctggcgcgaatgggcgtggaggcggtggcggaatctctgagggccagagccggccgctgcgatgggttcgccagactggtcgcgcaggcttaccgagacaccggatggcggtcaatggggcttgcgtaa

SEQ ID NO: 3 - protein, 220 aa, unidentified
  source 1..220: note = Uncultured bacterium RM44
MPILESVGFMKTLWESGGAQVALMESREETSHMVGILEGIAAELSWRPGTQLRDYQDRAAHLAVLVGSEIVGGLQIVTSPSADCLPYRLVWPEVCVPDGAAIADITILALRKEYRARFNLFWPLCVELWRHCVAEGATEMRLEATPDTLRLYRRIGWPLEVIGDLRLHWNEPCFLCRMGIVDVAGAMVVRALQSATYQAVLAGMSRPVASASPVATNSGL

SEQ ID NO: 4 - DNA, 70 bp, synthetic construct
  source 1..70: mol_type = other DNA; note = Synthetic primer
atgttttattgcgttaccgttcattcacaatactggagcaatccagtatgattccggggatccgtcgacc

SEQ ID NO: 5 - DNA, 70 bp, synthetic construct
  source 1..70: mol_type = other DNA; note = Synthetic primer
cgtacctctatcttgatttgcttgtttcattactcgtccttcacatttcctgtaggctggagctgcttcg

SEQ ID NO: 6 - DNA, 30 bp, synthetic construct
  source 1..30: mol_type = other DNA; note = Synthetic primer
gcgacgcgcgcaccttgcttaaccaggccc

SEQ ID NO: 7 - DNA, 27 bp, synthetic construct
  source 1..27: mol_type = other DNA; note = Synthetic primer
cgcatcttcgcgccaatccagaacacc

SEQ ID NO: 8 - DNA, 6700 bp, synthetic construct
  source 1..6700: mol_type = other DNA; note = Synthetic polynucleotide
ggggaattgtgagcggataacaattcccctgtagaaataattttgtttaactttaataaggagatataccatggtgaagaaggtttggcttaaccgttatcccgcggacgttccgacggagatcaaccctgaccgttatcaatctctggtagatatgtttgagcagtcggtcgcgcgctacgccgatcaacctgcgtttgtgaatatgggggaggtaatgaccttccgcaagctggaagaacgcagtcgcgcgtttgccgcttatttgcaacaagggttggggctgaagaaaggcgatcgcgttgcgttgatgatgcctaatttattgcaatatccggtggcgctgtttggcattttgcgtgccgggatgatcgtcgtaaacgttaacccgttgtataccccgcgtgagcttgagcatcagcttaacgatagcggcgcatcggcgattgttatcgtgtctaactttgctcacacactggaaaaagtggttgataaaaccgccgttcagcacgtaattctgacccgtatgggcgatcagctatctacggcaaaaggcacggtagtcaatttcgttgttaaatacatcaagcgtttggtgccgaaataccatctgccagatgccatttcatttcgtagcgcactgcataacggctaccggatgcagtacgtcaaacccgaactggtgccggaagatttagcttttctgcaatacaccggcggcaccactggtgtggcgaaaggcgcgatgctgactcaccgcaatatgctggcgaacctggaacaggttaacgcgacctatggtccgctgttgcatccgggcaaagagctggtggtgacggcgctgccgctgtatcacatttttgccctgaccattaactgcctgctgtttatcgaactgggtgggcagaacctgcttatcactaacccgcgcgatattccagggttggtaaaagagttagcgaaatatccgtttaccgctatcacgggcgttaacaccttgttcaatgcgttgctgaacaataaagagttccagcagctggatttctccagtctgcatctttccgcaggcggagggatgccagtgcagcaagtggtggcagagcgttgggtgaaactgacaggacagtatctgctggaaggctatggccttaccgagtgtgcgccgctggtcagcgttaacccatatgatattgattatcatagtggtagcatcggtttgccggtgccgtcgacggaagccaaactggtggatgatgatgataatgaagtaccaccgggtcaaccgggtgagctttgtgtcaaaggaccgcaggtgatgctgggttactggcagcgtccggatgctacagatgagatcatcaaaaatggctggttacacaccggcgacatcgcggtgatggatgaagaagggttcctgcgcattgtcgatcgtaaaaaagacatgattctggtttccggttttaacgtctatcccaacgagattgaagatgtcgtcatgcagcatcctggcgtacaggaagtcgcggctgttggcgtaccttccggctccagtggtgaagcggtgaaaatcttcgtagtgaaaaaagatccatcgcttaccgaagagtcactggtgaccttttgccgccgtcagctcacgggctacaaagtaccgaagctggtggagtttcgtgatgagttaccgaaatctaacgtcggaaaaattttgcgacgagaattacgtgacgaagcgcgcggcaaagtggacaataaagcctgaaagcttgcggccgcataatgcttaagtcgaacagaaagtaatcgtattgtacacggccgcataatcgaaattaatacgactcactataggggaattgtgagcggataacaattccccatcttagtatattagttaagtataagaaggagatatacatatgcgcccattacatccgattgattttatattcctgtcactagaaaaaagacaacagcctatgcatgtaggtggtttatttttgtttcagattcctgataacgccccagacacctttattcaagatctggtgaatgatatccggatatcaaaatcaatccctgttccaccattcaacaataaactgaatgggcttttttgggatgaagatgaagagtttgatttagatcatcattttcgtcatattgcactgcctcatcctggtcgtattcgtgaattgcttatttatatttcacaagagcacagtacgctgctagatcgggcaaagcccttgtggacctgcaatattattgaaggaattgaaggcaatcgttttgccatgtacttcaaaattcaccatgcgatggtcgatggcgttgctggtatgcggttaattgaaaaatcactctcccatgatgtaacagaaaaaagtatcgtgccaccttggtgtgttgagggaaaacgtgcaaagcgcttaagagaacctaaaacaggtaaaattaagaaaatcatgtctggtattaagagtcagcttcaggcgacacccacagtcattcaagagctttctcagacagtatttaaagatattggacgtaatcctgatcatgtttcaagctttcaggcgccttgttctattttgaatcagcgtgtgagctcatcgcgacgttttgcagcacagtcttttgacctagatcgttttcgtaatattgccaaatcgttgaatgtgaccattaatgatgttgtactagcggtatgttctggtgcattacgtgcgtatttgatgagtcataatagtttgccttcaaaaccattaattgccatggttccagcctctattcgcaatgacgattcagatgtcagcaaccgtattacgatgattctggcaaatttggcaacccacaaagatgatcctttacaacgtcttgaaattatccgccgtagtgttcaaaactcaaagcaacgcttcaaacgtatgaccagcgatcagattctaaattatagtgctgtcgtatatggccctgcaggactcaacataatttctggcatgatgccaaaacgccaagccttcaatctggttatttccaatgtgcctggcccaagagagccactttactggaatggtgccaaacttgatgcactctacccagcttcaattgtattagacggtcaagcattgaatattacaatgaccagttatttagataaacttgaagttggtttgattgcatgccgtaatgcattgccaagaatgcagaatttactgacacatttagaagaagaaattcaactatttgaaggcgtaattgcaaagcaggaagatattaaaacagccaattaaaaacaataaacttgattttttaatttatcagataaaactaaagggctaaattagccctcctaggctgctgccaccgctgagcaataactagcataaccccttggggcctctaaacgggtcttgaggggttttttgctgaaacctcaggcatttgagaagcacacggtcacactgcttccggtagtcaataaaccggtaaaccagcaatagacataagcggctatttaacgaccctgccctgaaccgacgaccgggtcatcgtggccggatcttgcggcccctcggcttgaacgaattgttagacattatttgccgactaccttggtgatctcgcctttcacgtagtggacaaattcttccaactgatctgcgcgcgaggccaagcgatcttcttcttgtccaagataagcctgtctagcttcaagtatgacgggctgatactgggccggcaggcgctccattgcccagtcggcagcgacatccttcggcgcgattttgccggttactgcgctgtaccaaatgcgggacaacgtaagcactacatttcgctcatcgccagcccagtcgggcggcgagttccatagcgttaaggtttcatttagcgcctcaaatagatcctgttcaggaaccggatcaaagagttcctccgccgctggacctaccaaggcaacgctatgttctcttgcttttgtcagcaagatagccagatcaatgtcgatcgtggctggctcgaagatacctgcaagaatgtcattgcgctgccattctccaaattgcagttcgcgcttagctggataacgccacggaatgatgtcgtcgtgcacaacaatggtgacttctacagcgcggagaatctcgctctctccaggggaagccgaagtttccaaaaggtcgttgatcaaagctcgccgcgttgtttcatcaagccttacggtcaccgtaaccagcaaatcaatatcactgtgtggcttcaggccgccatccactgcggagccgtacaaatgtacggccagcaacgtcggttcgagatggcgctcgatgacgccaactacctctgatagttgagtcgatacttcggcgatcaccgcttccctcatactcttcctttttcaatattattgaagcatttatcagggttattgtctcatgagcggatacatatttgaatgtatttagaaaaataaacaaatagctagctcactcggtcgctacgctccgggcgtgagactgcggcgggcgctgcggacacatacaaagttacccacagattccgtggataagcaggggactaacatgtgaggcaaaacagcagggccgcgccggtggcgtttttccataggctccgccctcctgccagagttcacataaacagacgcttttccggtgcatctgtgggagccgtgaggctcaaccatgaatctgacagtacgggcgaaacccgacaggacttaaagatccccaccgtttccggcgggtcgctccctcttgcgctctcctgttccgaccctgccgtttaccggatacctgttccgcctttctcccttacgggaagtgtggcgctttctcatagctcacacactggtatctcggctcggtgtaggtcgttcgctccaagctgggctgtaagcaagaactccccgttcagcccgactgctgcgccttatccggtaactgttcacttgagtccaacccggaaaagcacggtaaaacgccactggcagcagccattggtaactgggagttcgcagaggatttgtttagctaaacacgcggttgctcttgaagtgtgcgccaaagtccggctacactggaaggacagatttggttgctgtgctctgcgaaagccagttaccacggttaagcagttccccaactgacttaaccttcgatcaaaccacctccccaggtggttttttcgtttacagggcaaaagattacgcgcagaaaaaaaggatctcaagaagatcctttgatcttttctactgaaccgctctagatttcagtgcaatttatctcttcaaatgtagcacctgaagtcagccccatacgatataagttgtaattctcatgttagtcatgccccgcgcccaccggaaggagctgactgggttgaaggctctcaagggcatcggtcgagatcccggtgcctaatgagtgagctaacttacattaattgcgttgcgctcactgcccgctttccagtcgggaaacctgtcgtgccagctgcattaatgaatcggccaacgcgcggggagaggcggtttgcgtattgggcgccagggtggtttttcttttcaccagtgagacgggcaacagctgattgcccttcaccgcctggccctgagagagttgcagcaagcggtccacgctggtttgccccagcaggcgaaaatcctgtttgatggtggttaacggcgggatataacatgagctgtcttcggtatcgtcgtatcccactaccgagatgtccgcaccaacgcgcagcccggactcggtaatggcgcgcattgcgcccagcgccatctgatcgttggcaaccagcatcgcagtgggaacgatgccctcattcagcatttgcatggtttgttgaaaaccggacatggcactccagtcgccttcccgttccgctatcggctgaatttgattgcgagtgagatatttatgccagccagccagacgcagacgcgccgagacagaacttaatgggcccgctaacagcgcgatttgctggtgacccaatgcgaccagatgctccacgcccagtcgcgtaccgtcttcatgggagaaaataatactgttgatgggtgtctggtcagagacatcaagaaataacgccggaacattagtgcaggcagcttccacagcaatggcatcctggtcatccagcggatagttaatgatcagcccactgacgcgttgcgcgagaagattgtgcaccgccgctttacaggcttcgacgccgcttcgttctaccatcgacaccaccacgctggcacccagttgatcggcgcgagatttaatcgccgcgacaatttgcgacggcgcgtgcagggccagactggaggtggcaacgccaatcagcaacgactgtttgcccgccagttgttgtgccacgcggttgggaatgtaattcagctccgccatcgccgcttccactttttcccgcgttttcgcagaaacgtggctggcctggttcaccacgcgggaaacggtctgataagagacaccggcatactctgcgacatcgtataacgttactggtttcacattcaccaccctgaattgactctcttccgggcgctatcatgccataccgcgaaaggttttgcgccattcgatggtgtccgggatctcgacgctctcccttatgcgactcctgcattaggaaattaatacgactcactata

SEQ ID NO: 9 - DNA, 60 bp, synthetic construct
  source 1..60: mol_type = other DNA; note = Synthetic primer
  misc_feature 1..31: note = DNA
  misc_feature 32: note = RNA
  misc_feature 33..60: note = DNA
ctctagaaataatttaactttaagtaggagataggtacccatggcggacacgttattgat

SEQ ID NO: 10 - DNA, 58 bp, synthetic construct
  source 1..58: mol_type = other DNA; note = Synthetic primer
cttcgaattccatttaaattatttctagagtcattatgagtcatgatttactaaaggc

SEQ ID NO: 11 - DNA, 65 bp, synthetic construct
  source 1..65: mol_type = other DNA; note = Synthetic primer
ctctagaaataattttagttaagtataagaaggagatataccatggtgaagaaggtttggcttaa

SEQ ID NO: 12 - DNA, 51 bp, synthetic construct
  source 1..51: mol_type = other DNA; note = Synthetic primer
cttcgaattccatttaaattatttctagagttatcaggctttattgtccac

SEQ ID NO: 13 - DNA, 5733 bp, synthetic construct
  source 1..5733: mol_type = other DNA; note = Synthetic polynucleotide
actcaccagtcacagaaaagcatcttacggatggcatgacagtaagagaattatgcagtgctgccataaccatgagtgataacactgcggccaacttacttctgacaacgatcggaggaccgaaggagctaaccgcttttttgcacaacatgggggatcatgtaactcgccttgatcgttgggaaccggagctgaatgaagccataccaaacgacgagcgtgacaccacgatgcctgcagcaatggcaacaacgttgcgcaaactattaactggcgaactacttactctagcttcccggcaacaattaatagactggatggaggcggataaagttgcaggaccacttctgcgctcggcccttccggctggctggtttattgctgataaatctggagccggtgagcgtgggtctcgcggtatcattgcagcactggggccagatggtaagccctcccgtatcgtagttatctacacgacggggagtcaggcaactatggatgaacgaaatagacagatcgctgagataggtgcctcactgattaagcattggtaactgtcagaccaagtttactcatatatactttagattgatttaaaacttcatttttaatttaaaaggatctaggtgaagatcctttttgataatctcatgaccaaaatcccttaacgtgagttttcgttccactgagcgtcagaccccttaataagatgatcttcttgagatcgttttggtctgcgcgtaatctcttgctctgaaaacgaaaaaaccgccttgcagggcggtttttcgaaggttctctgagctaccaactctttgaaccgaggtaactggcttggaggagcgcagtcaccaaaacttgtcctttcagtttagccttaaccggcgcatgacttcaagactaactcctctaaatcaattaccagtggctgctgccagtggtgcttttgcatgtctttccgggttggactcaagacgatagttaccggataaggcgcagcggtcggactgaacggggggttcgtgcatacagtccagcttggagcgaactgcctacccggaactgagtgtcaggcgtggaatgagacaaacgcggccataacagcggaatgacaccggtaaaccgaaaggcaggaacaggagagcgcacgagggagccgccagggggaaacgcctggtatctttatagtcctgtcgggtttcgccaccactgatttgagcgtcagatttcgtgatgcttgtcaggggggcggagcctatggaaaaacggctttgccgcggccctctcacttccctgttaagtatcttcctggcatcttccaggaaatctccgccccgttcgtaagccatttccgctcgccgcagtcgaacgaccgagcgtagcgagtcagtgagcgaggaagcggaatatatcctgtatcacatattctgctgacgcaccggtgcagccttttttctcctgccacatgaagcacttcactgacaccctcatcagtgccaacatagtaagccagtatacactccgctagcgctgaggtctgcctcgtgaagaaggtgttgctgactcataccaggcctgaatcgccccatcatccagccagaaagtgagggagccacggttgatgagagctttgttgtaggtggaccagttggtgattttgaacttttgctttgccacggaacggtctgcgttgtcgggaagatgcgtgatctgatccttcaactcagcaaaagttcgatttattcaacaaagccacgttgtgtctcaaaatctctgatgttacattgcacaagataaaaatatatcatcatgaacaataaaactgtctgcttacataaacagtaatacaaggggtgttatgagccatattcaacgggaaacgtcttgctcgaggccgcgattaaattccaacatggatgctgatttatatgggtataaatgggctcgcgataatgtcgggcaatcaggtgcgacaatctatcgattgtatgggaagcccgatgcgccagagttgtttctgaaacatggcaaaggtagcgttgccaatgatgttacagatgagatggtcagactaaactggctgacggaatttatgcctcttccgaccatcaagcattttatccgtactcctgatgatgcatggttactcaccactgcgatccccgggaaaacagcattccaggtattagaagaatatcctgattcaggtgaaaatattgttgatgcgctggcagtgttcctgcgccggttgcattcgattcctgtttgtaattgtccttttaacagcgatcgcgtatttcgtctcgctcaggcgcaatcacgaatgaataacggtttggttgatgcgagtgattttgatgacgagcgtaatggctggcctgttgaacaagtctggaaagaaatgcataagcttttgccattctcaccggattcagtcgtcactcatggtgatttctcacttgataaccttatttttgacgaggggaaattaataggttgtattgatgttggacgagtcggaatcgcagaccgataccaggatcttgccatcctatggaactgcctcggtgagttttctccttcattacagaaacggctttttcaaaaatatggtattgataatcctgatatgaataaattgcagtttcatttgatgctcgatgagtttttctaatcagaattggttaattggttgtaacactggcagagcattacgctgacttgacgggacggcggctttgttgaataaatcgaacttttgctgagttgaaggatcagatcacgcatcttcccgacaacgcagaccgttccgtggcaaagcaaaagttcaaaatcaccaactggtccacctacaacaaagctctcatcaaccgtggctccctcactttctggctggatgatggggcgattcaggcctggtatgagtcagcaacaccttcttcacgaggcagacctcagcgctcaaagatgcaggggtaaaagctaaccgcatctttaccgacaaggcatccggcagttcaacagatcgggaagggctggatttgctgaggatgaaggtggaggaaggtgatgtcattctggtgaagaagctcgaccgtcttggccgcgacaccgccgacatgatccaactgataaaagagtttgatgctcagggtgtagcggttcggtttattgacgacgggatcagtaccgacggtgatatggggcaaatggtggtcaccatcctgtcggctgtggcacaggctgaacgccggaggatcctagagcgcacgaatgagggccgacaggaagcaaagctgaaaggaatcaaatttggccgcaggcgtaccgtggacaggaacgtcgtgctgacgcttcatcagaagggcactggtgcaacggaaattgctcatcagctcagtattgcccgctccacggtttataaaattcttgaagacgaaagggcctcgtgatacgcctatttttataggttaatgtcatgataataatggtttcttagacgtcttaattaatcaggagagcgttcaccgacaaacaacagataaaacgaaaggcccagtctttcgactgagcctttcgttttatttgatgcctggcagttccctactctcgcatggggagaccccacactaccatcggcgctacggcgtttcacttctgagttcggcatggggtcaggtgggaccaccgcgctactgccgccaggcaaattctgttttatcagaccgcttctgcgttctgatttaatctgtatcaggctgaaaatcttctctcatccgccaaaacagccaagctggagaccgtttaaactcaatgatgatgatgatgatggtcgacggcgctattcagatcctcttctgagatgagtttttgttcgggcccaagcttcgaattcccatatggtaccagctgcagatctcgagctcggatccatggtttattcctccttatttaatcgatacattaatatatacctctttaatttttaataataaagttaatcgataattccggtcgagtgcccacacagattgtctgataaattgttaaagagcagtgccgcttcgctttttctcagcggcgctgtttcctgtgtgaaattgttatccgctcacaattccacacattatacgagccggatgattaattgtcaacagctcatttcagaatatttgccagaaccgttatgatgtcggcgcaaaaaacattatccagaacgggagtgcgccttgagcgacacgaattatgcagtgatttacgacctgcacagccataccacagcttccgatggctgcctgacgccagaagcattggtgcaccgtgcagtcgatgataagctgtcaaaccagatcaattcgcgctaactcacattaattgcgttgcgctcactgcccgctttccagtcgggaaacctgtcgtgccagctgcattaatgaatcggccaacgcgcggggagaggcggtttgcgtattgggcgccagggtggtttttcttttcaccagtgagacgggcaacagctgattgcccttcaccgcctggccctgagagagttgcagcaagcggtccacgctggtttgccccagcaggcgaaaatcctgtttgatggtggttgacggcgggatataacatgagctgtcttcggtatcgtcgtatcccactaccgagatatccgcaccaacgcgcagcccggactcggtaatggcgcgcattgcgcccagcgccatctgatcgttggcaaccagcatcgcagtgggaacgatgccctcattcagcatttgcatggtttgttgaaaaccggacatggcactccagtcgccttcccgttccgctatcggctgaatttgattgcgagtgagatatttatgccagccagccagacgcagacgcgccgagacagaacttaatgggcccgctaacagcgcgatttgctggtgacccaatgcgaccagatgctccacgcccagtcgcgtaccgtcttcatgggagaaaataatactgttgatgggtgtctggtcagagacatcaagaaataacgccggaacattagtgcaggcagcttccacagcaatggcatcctggtcatccagcggatagttaatgatcagcccactgacgcgttgcgcgagaagattgtgcaccgccgctttacaggcttcgacgccgcttcgttctaccatcgacaccaccacgctggcacccagttgatcggcgcgagatttaatcgccgcgacaatttgcgacggcgcgtgcagggccagactggaggtggcaacgccaatcagcaacgactgtttgcccgccagttgttgtgccacgcggttgggaatgtaattcagctccgccatcgccgcttccactttttcccgcgttttcgcagaaacgtggctggcctggttcaccacgcgggaaacggtctgataagagacaccggcatactctgcgacatcgtataacgttactggtttcacattcaccaccctgaattgactctcttccgggcgctatcatgccataccgcgaaaggttttgcaccattcgatggtgtcaacgtaaatgcatgccgcttcgccttcgcgcgcgaattgatctgctgcctcgcgcgtttcggtgatgacggtgaaaacctctgacacatgcagctcccggagacggtcacagcttgtctgtaagcggatgccgggagcagacaagcccgtcagggcgcgtcagcgggtgttggcggggccggcctcg

SEQ ID NO: 14 - DNA, 36 bp, synthetic construct
  source 1..36: mol_type = other DNA; note = Synthetic primer
gggtcaatagcggccgccaattcgcgcgcgaaggcg

SEQ ID NO: 15 - DNA, 37 bp, synthetic construct
  source 1..37: mol_type = other DNA; note = Synthetic primer
tggcgcgcctcctagggcattacgctgacttgacggg

SEQ ID NO: 16 - DNA, 15179 bp, synthetic construct
  source 1..15179: mol_type = other DNA; note = Synthetic polynucleotide
ggccacgatgcgtccggcgtagaggatctgctcatgtttgacagcttatcatcgatgcataatgtgcctgtcaaatggacgaagcagggattctgcaaaccctatgctactccgtcaagccgtcaattgtctgattcgttaccaattatgacaacttgacggctacatcattcactttttcttcacaaccggcacggaactcgctcgggctggccccggtgcattttttaaatacccgcgagaaatagagttgatcgtcaaaaccaacattgcgaccgacggtggcgataggcatccgggtggtgctcaaaagcagcttcgcctggctgatacgttggtcctcgcgccagcttaagacgctaatccctaactgctggcggaaaagatgtgacagacgcgacggcgacaagcaaacatgctgtgcgacgctggcgatatcaaaattgctgtctgccaggtgatcgctgatgtactgacaagcctcgcgtacccgattatccatcggtggatggagcgactcgttaatcgcttccatgcgccgcagtaacaattgctcaagcagatttatcgccagcagctccgaatagcgcccttccccttgcccggcgttaatgatttgcccaaacaggtcgctgaaatgcggctggtgcgcttcatccgggcgaaagaaccccgtattggcaaatattgacggccagttaagccattcatgccagtaggcgcgcggacgaaagtaaacccactggtgataccattcgcgagcctccggatgacgaccgtagtgatgaatctctcctggcgggaacagcaaaatatcacccggtcggcaaacaaattctcgtccctgatttttcaccaccccctgaccgcgaatggtgagattgagaatataacctttcattcccagcggtcggtcgataaaaaaatcgagataaccgttggcctcaatcggcgttaaacccgccaccagatgggcattaaacgagtatcccggcagcaggggatcattttgcgcttcagccatacttttcatactcccgccattcagagaagaaaccaattgtccatattgcatcagacattgccgtcactgcgtcttttactggctcttctcgctaaccaaaccggtaaccccgcttattaaaagcattctgtaacaaagcgggaccaaagccatgacaaaaacgcgtaacaaaagtgtctataatcacggcagaaaagtccacattgattatttgcacggcgtcacactttgctatgccatagcatttttatccataagattagcggatcctacctgacgctttttatcgcaactctctactgtttctccatacccgtttttttgggctagcgaattcgagctcggtacccaagtcttaaactagacagaatagttgtaaactgaaatcagtccagttatgctgtgaaaaagcatactggacttttgttatggctaaagcaaactcttcattttctgaagtgcaaattgcccgtcgtattaaagaggggcgtggccaagggcatggtaaagactatattccatggctaacagtacaagaagttccttcttcaggtcgttcccaccgtatttattctcataagacgggacgagtccatcatttgctatctgacttagagcttgctgtttttctcagtcttgagtgggagagcagcgtgctagatatacgcgagcagttccccttattacctagtgataccaggcagattgcaatagatagtggtattaagcatcctgttattcgtggtgtagatcaggttatgtctactgattttttagtggactgcaaagatggtccttttgagcagtttgctattcaagtcaaacctgcagcagccttacaagacgagcgtaccttagaaaaactagaactagagcgtcgctattggcagcaaaagcaaattccttggttcatttttactgataaagaaataaatcccgtagtaaaagaaaatattgaatggctttattcagtgaaaacagaagaagtttctgcggagcttttagcacaactatccccattggcccatatcctgcaagaaaaaggagatgaaaacattatcaatgtctgtaagcaggttgatattgcttatgatttggagttaggcaaaacattgagtgagatacgagccttaaccgcaaatggttttattaagttcaatatttataagtctttcagggcaaataagtgtgcagatctctgtattagccaagtagtgaatatggaggagttgcgctatgtggcaaattaatgaggttgtgctatttgataatgatccgtatcgcattttggctatagaggatggccaagttgtctggatgcaaataagcgctgataaaggagttccacaagctagggctgagttgttgctaatgcagtatttagatgaaggccgcttagttagaactgatgacccttatgtacatcttgatttagaagagccgtctgtagattctgtcagcttccagaagcgcgaggaggattatcgaaaaattcttcctattattaatagtaaggatcgtttcgaccctaaagtcagaagcgaactcgttgagcatgtggtccaagaacataaggttactaaggctacagtttataagttgttacgccgttactggcagcgtggtcaaacgcctaatgcattaattcctgactacaaaaacagcggtgcaccaggggaaagacgttcagcgacaggaacagcaaagattggccgagccagagaatatggtaagggtgaaggaaccaaggtaacgcccgagattgaacgcctttttaggttgaccatagaaaagcacctgttaaatcaaaaaggtacaaagaccaccgttgcctatagacgatttgtggacttgtttgctcagtattttcctcgcattccccaagaggattacccaacactacgtcagtttcgttatttttatgatcgagaataccctaaagctcagcgcttaaagtctagagttaaagcaggggtatataaaaaagacgtacgacccttaagtagtacagccacttctcaggcgttaggccctgggagtcgttatgagattgatgccacgattgctgatatttatttagtggatcatcatgatcgccaaaaaatcataggaagaccaacgctttacattgtgattgatgtgtttagtcggatgatcacgggcttttatatcggctttgaaaatccgtcttatgtggtggcgatgcaggcttttgtaaatgcttgctctgacaaaacggccatttgtgcccagcatgatattgagattagtagctcagactggccgtgtgtaggtttgccagatgtgttgctagcggaccgtggcgaattaatgagtcatcaggtcgaagccttagtttctagttttaatgtgcgagtggaaagtgctccacctagacgtggcgatgctaaaggcatagtggaaagcacttttagaacactacaagccgagtttaagtcctttgcacctggcattgtagagggcagtcggatcaaaagccatggtgaaacagactataggttagatgcatctctgtcggtatttgagttcacacaaattattttgcgtacgatcttattcagaaataaccatctggtgatggataaatacgatcgagatgctgattttcctacagatttaccgtctattcctgtccagctatggcaatggggtatgcagcatcgtacaggtagtttaagggctgtggagcaagagcagttgcgagtagcgttactgcctcgccgaaaggtctctatttcttcatttggcgttaatttgtggggtttgtattactcggggtcagagattctgcgtgagggttggttgcagcggagcactgatatagctagacctcaacatttagaagcggcttatgacccagtgctggttgatacgatttatttgtttccgcaagttggcagccgtgtattttggcgctgtaatctgacggaacgtagtcggcagtttaaaggtctctcattttgggaggtttgggatatacaagcacaagaaaaacacaataaagccaatgcgaagcaggatgagttaactaaacgcagggagcttgaggcgtttattcagcaaaccattcagaaagcgaataagttaacgcccagtactactgagcccaaatcaacacgcattaagcagattaaaactaataaaaaagaagccgtgacctcggagcgtaaaaaacgtgcggagcatttgaagccaagctcttcaggtgatgaggctaaagttattcctttcaacgcagtggaagcggatgatcaagaagattacagcctacccacatacgtgcctgaattatttcaggatccaccagaaaaggatgagtcatgagtgctacccggattcaagcagtttatcgtgatacgggggtagaggcttatcgtgataatccttttatcgaggccttaccaccattacaagagtcagtgaatagtgctgcatcactgaaatcctctttacagcttacttcctctgacttgcaaaagtcccgtgttatcagagctcataccatttgtcgtattccagatgactattttcagccattaggtacgcatttgctactaagtgagcgtatttcggtcatgattcgaggtggctacgtaggcagaaatcctaaaacaggagatttacaaaagcatttacaaaatggttatgagcgtgttcaaacgggagagttggagacatttcgctttgaggaggcacgatctacggcacaaagcttattgttaattggttgttctggtagtgggaagacgacctctcttcatcgtattctagccacgtatcctcaggtgatttaccatcgtgaactcaatgtagagcaggtggtgtatttgaaaatagactgctcgcataatggttcgctaaaagaaatctgcttgaattttttcagagcgttggatcgagccttgggctcgaactatgagcgtcgttatggcttaaaacgtcatggtatagaaaccatgttggctttgatgtcgcaaatagccaatgcacatgctttagggttgttggttattgatgaaattcagcatttaagccgctctcgttcgggtggatctcaagagatgctgaacttttttgtgacgatggtgaatattattggcgtaccagtgatgttgattggtacccctaaagcacgagagatttttgaggctgatttgcggtctgcacgtagaggggcagggtttggagctatattctgggatcctatacaacaaacgcaacgtggaaagcccaatcaagagtggatcgcttttacggataatctttggcaattacagcttttacaacgcaaagatgcgctgttatcggatgaggtccgtgatgtgtggtatgagctaagccaaggagtgatggacattgtagtaaaactttttgtactcgctcagctccgtgcgctagctttaggcaatgagcgtattaccgctggtttattgcggcaagtgtatcaagatgagttaaagcctgtgcaccccatgctagaggcattacgctcgggtatcccagaacgcattgctcgttattctgatctagtcgttcccgagattgataaacggttaatccaacttcagctagatatcgcagcgatacaagaacaaacaccagaagaaaaagcccttcaagagttagataccgaagatcagcgtcatttatatctgatgctgaaagaggattacgattcaagcctgttaattcccactattaaaaaagcgtttagccagaatccaacgatgacaagacaaaagttactgcctcttgttttgcagtggttgatggaaggcgaaacggtagtgtcagaactagaaaagccctccaagagtaaaaaggtttcggctataaaggtagtcaagcccagcgactgggatagcttgcctgatacggatttacgttatatctattcacaacgccaacctgaaaaaaccatgcatgaacggttaaaagggaaaggggtaatagtggatatggcgagcttatttaaacaagcaggttagccatgagaaactttcctgttccgtactcgaatgagctgatttatagcactattgcacgggcaggcgtttatcaagggattgttagtcctaagcagctgttggatgaggtgtatggcaaccgcaaggtggtcgctaccttaggtctgccctcgcatttaggtgtgatagcaagacatctacatcaaacaggacgttacgctgttcagcagcttatttatgagcataccttattccctttatatgctccgtttgtaggcaaggagcgccgagacgaagctattcggttaatggagtaccaagcgcaaggtgcggtgcatttaatgctaggagtcgctgcttctagagttaagagcgataaccgctttagatactgccctgattgcgttgctcttcagctaaataggtatggggaagccttttggcaacgagattggtatttgcccgctttgccatattgtccaaaacacggtgctttagtcttctttgatagagctgtagatgatcaccgacatcaattttgggctttgggtcatactgagctgctttcagactaccccaaagactccctatctcaattaacagcactagctgcttatatagcccctctgttagatgctccacgagcgcaagagctttccccaagccttgagcagtggacgctgttttatcagcgcttagcgcaggatctagggctaaccaaaagcaagcacattcgtcatgacttggtggcggagagagtgaggcagacttttagtgatgaggcactagagaaactggatttaaagttggcagagaacaaggacacgtgttggctgaaaagtatattccgtaagcatagaaaagcctttagttatttacagcatagtattgtgtggcaagccttattgccaaaactaacggttatagaagcgctacagcaggcaagtgctcttactgagcactctataacgacaagacctgttagccagtctgtgcaacctaactctgaagatttatctgttaagcataaagactggcagcaactagtgcataaataccaaggaattaaggcggcaagacagtctttagagggtggggtgctatacgcttggctttaccgacatgacagggattggctagttcactggaatcaacagcatcaacaagagcgtctggcacccgcccctagagttgattggaaccaaagagatcgaattgctgtacgacaactattaagaatcataaagcgtctagatagtagccttgatcacccaagagcgacatcgagctggctgttaaagcaaactcctaacggaacctctcttgcaaaaaatctacagaaactgcctttggtagcgctttgcttaaagcgttactcagagagtgtggaagattatcaaattagacggattagccaagcttttattaagcttaaacaggaagatgttgagcttaggcgctggcgattattaagaagtgcaacgttatctaaagagcggataactgaggaagcacaaagattcttggaaatggtttatggggaagagtgagtggttaggctagctacatttaatgacaatgtgcaggttgtacatattggtcatttattccgtaactcgggtcataaggagtggcgtatttttgtttggtttaatccaatgcaagaacggaaatggactcgatttactcatttgcctttattaagtcgagctaaggtggttaacagtacaacaaagcaaataaataaggcggatcgtgtgattgagtttgaagcatcggatcttcaacgagccaaaataatcgattttcctaatctctcgtcctttgcttccgtacgcaacaaggatggagcgcagagttcatttatttacgaagctgaaacaccatatagcaagactcgttatcacatcccacagttagagctagctcggtcattatttttaggggatcctctagagtcgacctgcaggcatgcaagcttggctgttttggcggatgagagaagattttcagcctgatacagattaaatcagaacgcagaagcggtctgataaaacagaatttgcctggcggcagtagcgcggtggtcccacctgaccccatgccgaactcagaagtgaaacgccgtagcgccgatggtagtgtggggtctccccatgcgagagtagggaactgccaggcatcaaataaaacgaaaggctcagtcgaaagactgggcctttcgttttatctgttgtttgtcggtgaacgctctcctgagtaggacaaatccgccgggagcggatttgaacgttgcgaagcaacggcccggagggtggcgggcaggacgcccgccataaactgccaggcatcaaattaagcagaaggccatcctgacggatggcctttttgcgtttctacaaactcttttgtttatttttctaaatacattcaaatatgtatccgctcatgagacaataaccctgataaatgcttcaataatattgaaaaaggaagagtatgagtattcaacatttccgtgtcgcccttattcccttttttgcggcattttgccttcctgtttttgctcacccagaaacgctggtgaaagtaaaagatgctgaagatcagttgggtgcacgagtgggttacatcgaactggatctcaacagcggtaagatccttgagagttttcgccccgaagaacgttttccaatgatgagcacttttaaagttctgctatgtggcgcggtattatcccgtgttgacgccgggcaagagcaactcggtcgccgcatacactattctcagaatgacttggttgagtactcaccagtcacagaaaagcatcttacggatggcatgacagtaagagaattatgcagtgctgccataaccatgagtgataacactgcggccaacttacttctgacaacgatcggaggaccgaaggagctaaccgcttttttgcacaacatgggggatcatgtaactcgccttgatcgttgggaaccggagctgaatgaagccataccaaacgacgagcgtgacaccacgatgcctgcagcaatggcaacaacgttgcgcaaactattaactggcgaactacttactctagcttcccggcaacaattaatagactggatggaggcggataaagttgcaggaccacttctgcgctcggcccttccggctggctggtttattgctgataaatctggagccggtgagcgtgggtctcgcggtatcattgcagcactggggccagatggtaagccctcccgtatcgtagttatctacacgacggggagtcaggcaactatggatgaacgaaatagacagatcgctgagataggtgcctcactgattaagcattggtaactgtcagaccaagtttactcatatatactttagattgatttacgcgccctgtagcggcgcattaagcgcggcgggtgtggtggttacgcgcagcgtgaccgctacacttgccagcgccctagcgcccgctcctttcgctttcttcccttcctttctcgccacgttcgccgccggccagcctcgcagagcaggattcccgttgagcaccgccaggtgcgaataagggacagtgaagaaggaacacccgctcgcgggtgggcctacttcacctatcctgcccggcggcatcaccggcgccacaggtgcggttgctggcgcctatatcgccgacatcaccgatggggaagatcgggctcgccacttcgggctcatgagcgcttgtttcggcgtgggtatggtggcaggccccgtggccgggggactgttgggcgccatctccttgcatgcaccattccttgcggcggcggtgctcaacggcctcaacctactactgggctgcttcctaatgcaggagtcgcataagggagagcgtcgatccccgacagtaagacgggtaagcctgttgatgataccgctgccttactgggtgcattagccagtctgaatgacctgtcacgggataatccgaagtggtcagactggaaaatcagagggcaggaactgctgaacagcaaaaagtcagatagcaccacatagcagacccgccataaaacgccctgagaagcccgtgacgggcttttcttgtattatgggtagtttccttgcatgaatccataaaaggcgcctgtagtgccatttacccccattcactgccagagccgtgagcgcagcgaactgaatgtcacgaaaaagacagcgactcaggtgcctgatggtcggagacaaaaggaatattcagcgatttgcccgagcttgcgagggtgctacttaagcctttagggttttaaggtctgttttgtagaggagcaaacagcgtttgcgacatccttttgtaatactgcggaactgactaaagtagtgagttatacacagggctgggatctattctttttatctttttttattctttctttattctataaattataaccacttgaatataaacaaaaaaaacacacaaaggtctagcggaatttacagagggtctagcagaatttacaagttttccagcaaaggtctagcagaatttacagatacccacaactcaaaggaaaaggactagtaattatcattgactagcccatctcaattggtatagtgattaaaatcacctagaccaattgagatgtatgtctgaattagttgttttcaaagcaaatgaactagcgattagtcgctatgacttaacggagcatgaaaccaagctaattttatgctgtgtggcactactcaaccccacgattgaaaaccctacaaggaaagaacggacggtatcgttcacttataaccaatacgttcagatgatgaacatcagtagggaaaatgcttatggtgtattagctaaagcaaccagagagctgatgacgagaactgtggaaatcaggaatcctttggttaaaggctttgagattttccagtggacaaactatgccaagttctcaagcgaaaaattagaattagtttttagtgaagagatattgccttatcttttccagttaaaaaaattcataaaatataatctggaacatgttaagtcttttgaaaacaaatactctatgaggatttatgagtggttattaaaagaactaacacaaaagaaaactcacaaggcaaatatagagattagccttgatgaatttaagttcatgttaatgcttgaaaataactaccatgagtttaaaaggcttaaccaatgggttttgaaaccaataagtaaagatttaaacacttacagcaatatgaaattggtggttgataagcgaggccgcccgactgatacgttgattttccaagttgaactagatagacaaatggatctcgtaaccgaacttgagaacaaccagataaaaatgaatggtgacaaaataccaacaaccattacatcagattcctacctacataacggactaagaaaaacactacacgatgctttaactgcaaaaattcagctcaccagttttgaggcaaaatttttgagtgacatgcaaagtaagtatgatctcaatggttcgttctcatggctcacgcaaaaacaacgaaccacactagagaacatactggctaaatacggaaggatctgaggttcttatggctcttgtatctatcagtgaagcatcaagactaacaaacaaaagtagaacaactgttcaccgttacatatcaaagggaaaactgtccatatgcacagatgaaaacggtgtaaaaaagatagatacatcagagcttttacgagtttttggtgcatttaaagctgttcaccatgaacagatcgacaatgtaacagatgaacagcatgtaacacctaatagaacaggtgaaaccagtaaaacaaagcaactagaacatgaaattgaacacctgagacaacttgttacagctcaacagtcacacatagacagcctgaaacaggcgatgctgcttatcgaatcaaagctgccgacaacacgggagccagtgacgcctcccgtggggaaaaaatcatggcaattctggaagaaatagcgctttcagcctgtgggcggacaaaatagttgggaactgggaggggtggaaatggagtttttaaggattatttagggaagagtgacaaaatagatgggaactgggtgtagcgtcgtaagctaatacgaaaattaaaaatgacaaaatagtttggaactagatttcacttatctggttggtcgacactagtattaccctgttatccctagatttaaatgatatcggatcctagtaagccacgttttaattaatcagatgggtcaatagcggccgccaattcgcgcgcgaaggcgaagcggcatgcatttacgttgacaccatcgaatggtgcaaaacctttcgcggtatggcatgatagcgcccggaagagagtcaattcagggtggtgaatgtgaaaccagtaacgttatacgatgtcgcagagtatgccggtgtctcttatcagaccgtttcccgcgtggtgaaccaggccagccacgtttctgcgaaaacgcgggaaaaagtggaagcggcgatggcggagctgaattacattcccaaccgcgtggcacaacaactggcgggcaaacagtcgttgctgattggcgttgccacctccagtctggccctgcacgcgccgtcgcaaattgtcgcggcgattaaatctcgcgccgatcaactgggtgccagcgtggtggtgtcgatggtagaacgaagcggcgtcgaagcctgtaaagcggcggtgcacaatcttctcgcgcaacgcgtcagtgggctgatcattaactatccgctggatgaccaggatgccattgctgtggaagctgcctgcactaatgttccggcgttatttcttgatgtctctgaccagacacccatcaacagtattattttctcccatgaagacggtacgcgactgggcgtggagcatctggtcgcattgggtcaccagcaaatcgcgctgttagcgggcccattaagttctgtctcggcgcgtctgcgtctggctggctggcataaatatctcactcgcaatcaaattcagccgatagcggaacgggaaggcgactggagtgccatgtccggttttcaacaaaccatgcaaatgctgaatgagggcatcgttcccactgcgatgctggttgccaacgatcagatggcgctgggcgcaatgcgcgccattaccgagtccgggctgcgcgttggtgcggatatctcggtagtgggatacgacgataccgaagacagctcatgttatatcccgccgtcaaccaccatcaaacaggattttcgcctgctggggcaaaccagcgtggaccgcttgctgcaactctctcagggccaggcggtgaagggcaatcagctgttgcccgtctcactggtgaaaagaaaaaccaccctggcgcccaatacgcaaaccgcctctccccgcgcgttggccgattcattaatgcagctggcacgacaggtttcccgactggaaagcgggcagtgagcgcaacgcaattaatgtgagttagcgcgaattgatctggtttgacagcttatcatcgactgcacggtgcaccaatgcttctggcgtcaggcagccatcggaagctgtggtatggctgtgcaggtcgtaaatcactgcataattcgtgtcgctcaaggcgcactcccgttctggataatgttttttgcgccgacatcataacggttctggcaaatattctgaaatgagctgttgacaattaatcatccggctcgtataatgtgtggaattgtgagcggataacaatttcacacaggaaacagcgccgctgagaaaaagcgaagcggcactgctctttaacaatttatcagacaatctgtgtgggcactcgaccggaattatcgattaactttattattaaaaattaaagaggtatatattaatgtatcgattaaataaggaggaataaaccatggcggacacgttattgattctgggtgatagcctgagcgccgggtatcgaatgtctgccagcgcggcctggcctgccttgttgaatgataagtggcagagtaaaacgtcggtagttaatgccagcatcagcggcgacacctcgcaacaaggactggcgcgccttccggctctgctgaaacagcatcagccgcgttgggtgctggttgaactgggcggcaatgacggtttgcgtggttttcagccacagcaaaccgagcaaacgctgcgccagattttgcaggatgtcaaagccgccaacgctgaaccattgttaatgcaaatacgtctgcctgcaaactatggtcgccgttataatgaagcctttagcgccatttaccccaaactcgccaaagagtttgatgttccgctgctgcccttttttatggaagaggtctacctcaagccacaatggatgcaggatgacggtattcatcccaaccgcgacgcccagccgtttattgccgactggatggcgaagcagttgcagcctttagtaaatcatgactcataatgactctagaaataatttaaatggaattcgaagcttgggcccgaacaaaaactcatctcagaagaggatctgaatagcgccgtcgaccatcatcatcatcatcattgagtttaaacggtctccagcttggctgttttggcggatgagagaagattttcagcctgatacagattaaatcagaacgcagaagcggtctgataaaacagaatttgcctggcggcagtagcgcggtggtcccacctgaccccatgccgaactcagaagtgaaacgccgtagcgccgatggtagtgtggggtctccccatgcgagagtagggaactgccaggcatcaaataaaacgaaaggctcagtcgaaagactgggcctttcgttttatctgttgtttgtcggtgaacgctctcctgattaattaagacgtcccgtcaagtcagcgtaatgccctaggaggcgcgccacggccgcgtcgaccccacgcccctctttaatacgacgggcaatttgcacttcagaaaatgaagagtttgctttagccataacaaaagtccagtatgctttttcacagcataactggactgatttcagtttacaactattctgtctagtttaagactttattgtcatagtttagatctattttgttcagtttaagactttattgtccgcccaca

SEQ ID NO: 17 - DNA, 17683 bp, synthetic construct
  source 1..17683: mol_type = other DNA; note = Synthetic polynucleotide
ggccacgatgcgtccggcgtagaggatctgctcatgtttgacagcttatcatcgatgcataatgtgcctgtcaaatggacgaagcagggattctgcaaaccctatgctactccgtcaagccgtcaattgtctgattcgttaccaattatgacaacttgacggctacatcattcactttttcttcacaaccggcacggaactcgctcgggctggccccggtgcattttttaaatacccgcgagaaatagagttgatcgtcaaaaccaacattgcgaccgacggtggcgataggcatccgggtggtgctcaaaagcagcttcgcctggctgatacgttggtcctcgcgccagcttaagacgctaatccctaactgctggcggaaaagatgtgacagacgcgacggcgacaagcaaacatgctgtgcgacgctggcgatatcaaaattgctgtctgccaggtgatcgctgatgtactgacaagcctcgcgtacccgattatccatcggtggatggagcgactcgttaatcgcttccatgcgccgcagtaacaattgctcaagcagatttatcgccagcagctccgaatagcgcccttccccttgcccggcgttaatgatttgcccaaacaggtcgctgaaatgcggctggtgcgcttcatccgggcgaaagaaccccgtattggcaaatattgacggccagttaagccattcatgccagtaggcgcgcggacgaaagtaaacccactggtgataccattcgcgagcctccggatgacgaccgtagtgatgaatctctcctggcgggaacagcaaaatatcacccggtcggcaaacaaattctcgtccctgatttttcaccaccccctgaccgcgaatggtgagattgagaatataacctttcattcccagcggtcggtcgataaaaaaatcgagataaccgttggcctcaatcggcgttaaacccgccaccagatgggcattaaacgagtatcccggcagcaggggatcattttgcgcttcagccatacttttcatactcccgccattcagagaagaaaccaattgtccatattgcatcagacattgccgtcactgcgtcttttactggctcttctcgctaaccaaaccggtaaccccgcttattaaaagcattctgtaacaaagcgggaccaaagccatgacaaaaacgcgtaacaaaagtgtctataatcacggcagaaaagtccacattgattatttgcacggcgtcacactttgctatgccatagcatttttatccataagattagcggatcctacctgacgctttttatcgcaactctctactgtttctccatacccgtttttttgggctagcgaattcgagctcggtacccaagtcttaaactagacagaatagttgtaaactgaaatcagtccagttatgctgtgaaaaagcatactggacttttgttatggctaaagcaaactcttcattttctgaagtgcaaattgcccgtcgtattaaagaggggcgtggccaagggcatggtaaagactatattccatggctaacagtacaagaagttccttcttcaggtcgttcccaccgtatttattctcataagacgggacgagtccatcatttgctatctgacttagagcttgctgtttttctcagtcttgagtgggagagcagcgtgctagatatacgcgagcagttccccttattacctagtgataccaggcagattgcaatagatagtggtattaagcatcctgttattcgtggtgtagatcaggttatgtctactgattttttagtggactgcaaagatggtccttttgagcagtttgctattcaagtcaaacctgcagcagccttacaagacgagcgtaccttagaaaaactagaactagagcgtcgctattggcagcaaaagcaaattccttggttcatttttactgataaagaaataaatcccgtagtaaaagaaaatattgaatggctttattcagtgaaaacagaagaagtttctgcggagcttttagcacaactatccccattggcccatatcctgcaagaaaaaggagatgaaaacattatcaatgtctgtaagcaggttgatattgcttatgatttggagttaggcaaaacattgagtgagatacgagccttaaccgcaaatggttttattaagttcaatatttataagtctttcagggcaaataagtgtgcagatctctgtattagccaagtagtgaatatggaggagttgcgctatgtggcaaattaatgaggttgtgctatttgataatgatccgtatcgcattttggctatagaggatggccaagttgtctggatgcaaataagcgctgataaaggagttccacaagctagggctgagttgttgctaatgcagtatttagatgaaggccgcttagttagaactgatgacccttatgtacatcttgatttagaagagccgtctgtagattctgtcagcttccagaagcgcgaggaggattatcgaaaaattcttcctattattaatagtaaggatcgtttcgaccctaaagtcagaagcgaactcgttgagcatgtggtccaagaacataaggttactaaggctacagtttataagttgttacgccgttactggcagcgtggtcaaacgcctaatgcattaattcctgactacaaaaacagcggtgcaccaggggaaagacgttcagcgacaggaacagcaaagattggccgagccagagaatatggtaagggtgaaggaaccaaggtaacgcccgagattgaacgcctttttaggttgaccatagaaaagcacctgttaaatcaaaaaggtacaaagaccaccgttgcctatagacgatttgtggacttgtttgctcagtattttcctcgcattccccaagaggattacccaacactacgtcagtttcgttatttttatgatcgagaataccctaaagctcagcgcttaaagtctagagttaaagcaggggtatataaaaaagacgtacgacccttaagtagtacagccacttctcaggcgttaggccctgggagtcgttatgagattgatgccacgattgctgatatttatttagtggatcatcatgatcgccaaaaaatcataggaagaccaacgctttacattgtgattgatgtgtttagtcggatgatcacgggcttttatatcggctttgaaaatccgtcttatgtggtggcgatgcaggcttttgtaaatgcttgctctgacaaaacggccatttgtgcccagcatgatattgagattagtagctcagactggccgtgtgtaggtttgccagatgtgttgctagcggaccgtggcgaattaatgagtcatcaggtcgaagccttagtttctagttttaatgtgcgagtggaaagtgctccacctagacgtggcgatgctaaaggcatagtggaaagcacttttagaacactacaagccgagtttaagtcctttgcacctggcattgtagagggcagtcggatcaaaagccatggtgaaacagactataggttagatgcatctctgtcggtatttgagttcacacaaattattttgcgtacgatcttattcagaaataaccatctggtgatggataaatacgatcgagatgctgattttcctacagatttaccgtctattcctgtccagctatggcaatggggtatgcagcatcgtacaggtagtttaagggctgtggagcaagagcagttgcgagtagcgttactgcctcgccgaaaggtctctatttcttcatttggcgttaatttgtggggtttgtattactcggggtcagagattctgcgtgagggttggttgcagcggagcactgatatagctagacctcaacatttagaagcggcttatgacccagtgctggttgatacgatttatttgtttccgcaagttggcagccgtgtattttggcgctgtaatctgacggaacgtagtcggcagtttaaaggtctctcattttgggaggtttgggatatacaagcacaagaaaaacacaataaagccaatgcgaagcaggatgagttaactaaacgcagggagcttgaggcgtttattcagcaaaccattcagaaagcgaataagttaacgcccagtactactgagcccaaatcaacacgcattaagcagattaaaactaataaaaaagaagccgtgacctcggagcgtaaaaaacgtgcggagcatttgaagccaagctcttcaggtgatgaggctaaagttattcctttcaacgcagtggaagcggatgatcaagaagattacagcctacccacatacgtgcctgaattatttcaggatccaccagaaaaggatgagtcatgagtgctacccggattcaagcagtttatcgtgatacgggggtagaggcttatcgtgataatccttttatcgaggccttaccaccattacaagagtcagtgaatagtgctgcatcactgaaatcctctttacagcttacttcctctgacttgcaaaagtcccgtgttatcagagctcataccatttgtcgtattccagatgactattttcagccattaggtacgcatttgctactaagtgagcgtatttcggtcatgattcgaggtggctacgtaggcagaaatcctaaaacaggagatttacaaaagcatttacaaaatggttatgagcgtgttcaaacgggagagttggagacatttcgctttgaggaggcacgatctacggcacaaagcttattgttaattggttgttctggtagtgggaagacgacctctcttcatcgtattctagccacgtatcctcaggtgatttaccatcgtgaactcaatgtagagcaggtggtgtatttgaaaatagactgctcgcataatggttcgctaaaagaaatctgcttgaattttttcagagcgttggatcgagccttgggctcgaactatgagcgtcgttatggcttaaaacgtcatggtatagaaaccatgttggctttgatgtcgcaaatagccaatgcacatgctttagggttgttggttattgatgaaattcagcatttaagccgctctcgttcgggtggatctcaagagatgctgaacttttttgtgacgatggtgaatattattggcgtaccagtgatgttgattggtacccctaaagcacgagagatttttgaggctgatttgcggtctgcacgtagaggggcagggtttggagctatattctgggatcctatacaacaaacgcaacgtggaaagcccaatcaagagtggatcgcttttacggataatctttggcaattacagcttttacaacgcaaagatgcgctgttatcggatgaggtccgtgatgtgtggtatgagctaagccaaggagtgatggacattgtagtaaaactttttgtactcgctcagctccgtgcgctagctttaggcaatgagcgtattaccgctggtttattgcggcaagtgtatcaagatgagttaaagcctgtgcaccccatgctagaggcattacgctcgggtatcccagaacgcattgctcgttattctgatctagtcgttcccgagattgataaacggttaatccaacttcagctagatatcgcagcgatacaagaacaaacaccagaagaaaaagcccttcaagagttagataccgaagatcagcgtcatttatatctgatgctgaaagaggattacgattcaagcctgttaattcccactattaaaaaagcgtttagccagaatccaacgatgacaagacaaaagttactgcctcttgttttgcagtggttgatggaaggcgaaacggtagtgtcagaactagaaaagccctccaagagtaaaaaggtttcggctataaaggtagtcaagcccagcgactgggatagcttgcctgatacggatttacgttatatctattcacaacgccaacctgaaaaaaccatgcatgaacggttaaaagggaaaggggtaatagtggatatggcgagcttatttaaacaagcaggttagccatgagaaactttcctgttccgtactcgaatgagctgatttatagcactattgcacgggcaggcgtttatcaagggattgttagtcctaagcagctgttggatgaggtgtatggcaaccgcaaggtggtcgctaccttaggtctgccctcgcatttaggtgtgatagcaagacatctacatcaaacaggacgttacgctgttcagcagcttatttatgagcataccttattccctttatatgctccgtttgtaggcaaggagcgccgagacgaagctattcggttaatggagtaccaagcgcaaggtgcggtgcatttaatgctaggagtcgctgcttctagagttaagagcgataaccgctttagatactgccctgattgcgttgctcttcagctaaataggtatggggaagccttttggcaacgagattggtatttgcccgctttgccatattgtccaaaacacggtgctttagtcttctttgatagagctgtagatgatcaccgacatcaattttgggctttgggtcatactgagctgctttcagactaccccaaagactccctatctcaattaacagcactagctgcttatatagcccctctgttagatgctccacgagcgcaagagctttccccaagccttgagcagtggacgctgttttatcagcgcttagcgcaggatctagggctaaccaaaagcaagcacattcgtcatgacttggtggcggagagagtgaggcagacttttagtgatgaggcactagagaaactggatttaaagttggcagagaacaaggacacgtgttggctgaaaagtatattccgtaagcatagaaaagcctttagttatttacagcatagtattgtgtggcaagccttattgccaaaactaacggttatagaagcgctacagcaggcaagtgctcttactgagcactctataacgacaagacctgttagccagtctgtgcaacctaactctgaagatttatctgttaagcataaagactggcagcaactagtgcataaataccaaggaattaaggcggcaagacagtctttagagggtggggtgctatacgcttggctttaccgacatgacagggattggctagttcactggaatcaacagcatcaacaagagcgtctggcacccgcccctagagttgattggaaccaaagagatcgaattgctgtacgacaactattaagaatcataaagcgtctagatagtagccttgatcacccaagagcgacatcgagctggctgttaaagcaaactcctaacggaacctctcttgcaaaaaatctacagaaactgcctttggtagcgctttgcttaaagcgttactcagagagtgtggaagattatcaaattagacggattagccaagcttttattaagcttaaacaggaagatgttgagcttaggcgctggcgattattaagaagtgcaacgttatctaaagagcggataactgaggaagcacaaagattcttggaaatggtttatggggaagagtgagtggttaggctagctacatttaatgacaatgtgcaggttgtacatattggtcatttattccgtaactcgggtcataaggagtggcgtatttttgtttggtttaatccaatgcaagaacggaaatggactcgatttactcatttgcctttattaagtcgagctaaggtggttaacagtacaacaaagcaaataaataaggcggatcgtgtgattgagtttgaagcatcggatcttcaacgagccaaaataatcgattttcctaatctctcgtcctttgcttccgtacgcaacaaggatggagcgcagagttcatttatttacgaagctgaaacaccatatagcaagactcgttatcacatcccacagttagagctagctcggtcattatttttaggggatcctctagagtcgacctgcaggcatgcaagcttggctgttttggcggatgagagaagattttcagcctgatacagattaaatcagaacgcagaagcggtctgataaaacagaatttgcctggcggcagtagcgcggtggtcccacctgaccccatgccgaactcagaagtgaaacgccgtagcgccgatggtagtgtggggtctccccatgcgagagtagggaactgccaggcatcaaataaaacgaaaggctcagtcgaaagactgggcctttcgttttatctgttgtttgtcggtgaacgctctcctgagtaggacaaatccgccgggagcggatttgaacgttgcgaagcaacggcccggagggtggcgggcaggacgcccgccataaactgccaggcatcaaattaagcagaaggccatcctgacggatggcctttttgcgtttctacaaactcttttgtttatttttctaaatacattcaaatatgtatccgctcatgagacaataaccctgataaatgcttcaataatattgaaaaaggaagagtatgagtattcaacatttccgtgtcgcccttattcccttttttgcggcattttgccttcctgtttttgctcacccagaaacgctggtgaaagtaaaagatgctgaagatcagttgggtgcacgagtgggttacatcgaactggatctcaacagcggtaagatccttgagagttttcgccccgaagaacgttttccaatgatgagcacttttaaagttctgctatgtggcgcggtattatcccgtgttgacgccgggcaagagcaactcggtcgccgcatacactattctcagaatgacttggttgagtactcaccagtcacagaaaagcatcttacggatggcatgacagtaagagaattatgcagtgctgccataaccatgagtgataacactgcggccaacttacttctgacaacgatcggaggaccgaaggagctaaccgcttttttgcacaacatgggggatcatgtaactcgccttgatcgttgggaaccggagctgaatgaagccataccaaacgacgagcgtgacaccacgatgcctgcagcaatggcaacaacgttgcgcaaactattaactggcgaactacttactctagcttcccggcaacaattaatagactggatggaggcggataaagttgcaggaccacttctgcgctcggcccttccggctggctggtttattgctgataaatctggagccggtgagcgtgggtctcgcggtatcattgcagcactggggccagatggtaagccctcccgtatcgtagttatctacacgacggggagtcaggcaactatggatgaacgaaatagacagatcgctgagataggtgcctcactgattaagcattggtaactgtcagaccaagtttactcatatatactttagattgatttacgcgccctgtagcggcgcattaagcgcggcgggtgtggtggttacgcgcagcgtgaccgctacacttgccagcgccctagcgcccgctcctttcgctttcttcccttcctttctcgccacgttcgccgccggccagcctcgcagagcaggattcccgttgagcaccgccaggtgcgaataagggacagtgaagaaggaacacccgctcgcgggtgggcctacttcacctatcctgcccggcggcatcaccggcgccacaggtgcggttgctggcgcctatatcgccgacatcaccgatggggaagatcgggctcgccacttcgggctcatgagcgcttgtttcggcgtgggtatggtggcaggccccgtggccgggggactgttgggcgccatctccttgcatgcaccattccttgcggcggcggtgctcaacggcctcaacctactactgggctgcttcctaatgcaggagtcgcataagggagagcgtcgatccccgacagtaagacgggtaagcctgttgatgataccgctgccttactgggtgcattagccagtctgaatgacctgtcacgggataatccgaagtggtcagactggaaaatcagagggcaggaactgctgaacagcaaaaagtcagatagcaccacatagcagacccgccataaaacgccctgagaagcccgtgacgggcttttcttgtattatgggtagtttccttgcatgaatccataaaaggcgcctgtagtgccatttacccccattcactgccagagccgtgagcgcagcgaactgaatgtcacgaaaaagacagcgactcaggtgcctgatggtcggagacaaaaggaatattcagcgatttgcccgagcttgcgagggtgctacttaagcctttagggttttaaggtctgttttgtagaggagcaaacagcgtttgcgacatccttttgtaatactgcggaactgactaaagtagtgagttatacacagggctgggatctattctttttatctttttttattctttctttattctataaattataaccacttgaatataaacaaaaaaaacacacaaaggtctagcggaatttacagagggtctagcagaatttacaagttttccagcaaaggtctagcagaatttacagatacccacaactcaaaggaaaaggactagtaattatcattgactagcccatctcaattggtatagtgattaaaatcacctagaccaattgagatgtatgtctgaattagttgttttcaaagcaaatgaactagcgattagtcgctatgacttaacggagcatgaaaccaagctaattttatgctgtgtggcactactcaaccccacgattgaaaaccctacaaggaaagaacggacggtatcgttcacttataaccaatacgttcagatgatgaacatcagtagggaaaatgcttatggtgtattagctaaagcaaccagagagctgatgacgagaactgtggaaatcaggaatcctttggttaaaggctttgagattttccagtggacaaactatgccaagttctcaagcgaaaaattagaattagtttttagtgaagagatattgccttatcttttccagttaaaaaaattcataaaatataatctggaacatgttaagtcttttgaaaacaaatactctatgaggatttatgagtggttattaaaagaactaacacaaaagaaaactcacaaggcaaatatagagattagccttgatgaatttaagttcatgttaatgcttgaaaataactaccatgagtttaaaaggcttaaccaatgggttttgaaaccaataagtaaagatttaaacacttacagcaatatgaaattggtggttgataagcgaggccgcccgactgatacgttgattttccaagttgaactagatagacaaatggatctcgtaaccgaacttgagaacaaccagataaaaatgaatggtgacaaaataccaacaaccattacatcagattcctacctacataacggactaagaaaaacactacacgatgctttaactgcaaaaattcagctcaccagttttgaggcaaaatttttgagtgacatgcaaagtaagtatgatctcaatggttcgttctcatggctcacgcaaaaacaacgaaccacactagagaacatactggctaaatacggaaggatctgaggttcttatggctcttgtatctatcagtgaagcatcaagactaacaaacaaaagtagaacaactgttcaccgttacatatcaaagggaaaactgtccatatgcacagatgaaaacggtgtaaaaaagatagatacatcagagcttttacgagtttttggtgcatttaaagctgttcaccatgaacagatcgacaatgtaacagatgaacagcatgtaacacctaatagaacaggtgaaaccagtaaaacaaagcaactagaacatgaaattgaacacctgagacaacttgttacagctcaacagtcacacatagacagcctgaaacaggcgatgctgcttatcgaatcaaagctgccgacaacacgggagccagtgacgcctcccgtggggaaaaaatcatggcaattctggaagaaatagcgctttcagcctgtgggcggacaaaatagttgggaactgggaggggtggaaatggagtttttaaggattatttagggaagagtgacaaaatagatgggaactgggtgtagcgtcgtaagctaatacgaaaattaaaaatgacaaaatagtttggaactagatttcacttatctggttggtcgacactagtattaccctgttatccctagatttaaatgatatcggatcctagtaagccacgttttaattaatcagatgggtcaatagcggccgccaattcgcgcgcgaaggcgaagcggcatgcatttacgttgacaccatcgaatggtgcaaaacctttcgcggtatggcatgatagcgcccggaagagagtcaattcagggtggtgaatgtgaaaccagtaacgttatacgatgtcgcagagtatgccggtgtctcttatcagaccgtttcccgcgtggtgaaccaggccagccacgtttctgcgaaaacgcgggaaaaagtggaagcggcgatggcggagctgaattacattcccaaccgcgtggcacaacaactggcgggcaaacagtcgttgctgattggcgttgccacctccagtctggccctgcacgcgccgtcgcaaattgtcgcggcgattaaatctcgcgccgatcaactgggtgccagcgtggtggtgtcgatggtagaacgaagcggcgtcgaagcctgtaaagcggcggtgcacaatcttctcgcgcaacgcgtcagtgggctgatcattaactatccgctggatgaccaggatgccattgctgtggaagctgcctgcactaatgttccggcgttatttcttgatgtctctgaccagacacccatcaacagtattattttctcccatgaagacggtacgcgactgggcgtggagcatctggtcgcattgggtcaccagcaaatcgcgctgttagcgggcccattaagttctgtctcggcgcgtctgcgtctggctggctggcataaatatctcactcgcaatcaaattcagccgatagcggaacgggaaggcgactggagtgccatgtccggttttcaacaaaccatgcaaatgctgaatgagggcatcgttcccactgcgatgctggttgccaacgatcagatggcgctgggcgcaatgcgcgccattaccgagtccgggctgcgcgttggtgcggatatctcggtagtgggatacgacgataccgaagacagctcatgttatatcccgccgtcaaccaccatcaaacaggattttcgcctgctggggcaaaccagcgtggaccgcttgctgcaactctctcagggccaggcggtgaagggcaatcagctgttgcccgtctcactggtgaaaagaaaaaccaccctggcgcccaatacgcaaaccgcctctccccgcgcgttggccgattcattaatgcagctggcacgacaggtttcccgactggaaagcgggcagtgagcgcaacgcaattaatgtgagttagcgcgaattgatctggtttgacagcttatcatcgactgcacggtgcaccaatgcttctggcgtcaggcagccatcggaagctgtggtatggctgtgcaggtcgtaaatcactgcataattcgtgtcgctcaaggcgcactcccgttctggataatgttttttgcgccgacatcataacggttctggcaaatattctgaaatgagctgttgacaattaatcatccggctcgtataatgtgtggaattgtgagcggataacaatttcacacaggaaacagcgccgctgagaaaaagcgaagcggcactgctctttaacaatttatcagacaatctgtgtgggcactcgaccggaattatcgattaactttattattaaaaattaaagaggtatatattaatgtatcgattaaataaggaggaataaaccatggcggacacgttattgattctgggtgatagcctgagcgccgggtatcgaatgtctgccagcgcggcctggcctgccttgttgaatgataagtggcagagtaaaacgtcggtagttaatgccagcatcagcggcgacacctcgcaacaaggactggcgcgccttccggctctgctgaaacagcatcagccgcgttgggtgctggttgaactgggcggcaatgacggtttgcgtggttttcagccacagcaaaccgagcaaacgctgcgccagattttgcaggatgtcaaagccgccaacgctgaaccattgttaatgcaaatacgtctgcctgcaaactatggtcgccgttataatgaagcctttagcgccatttaccccaaactcgccaaagagtttgatgttccgctgctgcccttttttatggaagaggtctacctcaagccacaatggatgcaggatgacggtattcatcccaaccgcgacgcccagccgtttattgccgactggatggcgaagcagttgcagcctttagtaaatcatgactcataatgactctagaaataattttagttaagtataagaaggagatataccatggtgaagaaggtttggcttaaccgttatcccgcggacgttccgacggagatcaaccctgaccgttatcaatctctggtagatatgtttgagcagtcggtcgcgcgctacgccgatcaacctgcgtttgtgaatatgggggaggtaatgaccttccgcaagctggaagaacgcagtcgcgcgtttgccgcttatttgcaacaagggttggggctgaagaaaggcgatcgcgttgcgttgatgatgcctaatttattgcaatatccggtggcgctgtttggcattttgcgtgccgggatgatcgtcgtaaacgttaacccgttgtataccccgcgtgagcttgagcatcagcttaacgatagcggcgcatcggcgattgttatcgtgtctaactttgctcacacactggaaaaagtggttgataaaaccgccgttcagcacgtaattctgacccgtatgggcgatcagctatctacggcaaaaggcacggtagtcaatttcgttgttaaatacatcaagcgtttggtgccgaaataccatctgccagatgccatttcatttcgtagcgcactgcataacggctaccggatgcagtacgtcaaacccgaactggtgccggaagatttagcttttctgcaatacaccggcggcaccactggtgtggcgaaaggcgcgatgctgactcaccgcaatatgctggcgaacctggaacaggttaacgcgacctatggtccgctgttgcatccgggcaaagagctggtggtgacggcgctgccgctgtatcacatttttgccctgaccattaactgcctgctgtttatcgaactgggtgggcagaacctgcttatcactaacccgcgcgatattccagggttggtaaaagagttagcgaaatatccgtttaccgctatcacgggcgttaacaccttgttcaatgcgttgctgaacaataaagagttccagcagctggatttctccagtctgcatctttccgcaggcggagggatgccagtgcagcaagtggtggcagagcgttgggtgaaactgacaggacagtatctgctggaaggctatggccttaccgagtgtgcgccgctggtcagcgttaacccatatgatattgattatcatagtggtagcatcggtttgccggtgccgtcgacggaagccaaactggtggatgatgatgataatgaagtaccaccgggtcaaccgggtgagctttgtgtcaaaggaccgcaggtgatgctgggttactggcagcgtccggatgctacagatgagatcatcaaaaatggctggttacacaccggcgacatcgcggtgatggatgaagaagggttcctgcgcattgtcgatcgtaaaaaagacatgattctggtttccggttttaacgtctatcccaacgagattgaagatgtcgtcatgcagcatcctggcgtacaggaagtcgcggctgttggcgtaccttccggctccagtggtgaagcggtgaaaatcttcgtagtgaaaaaagatccatcgcttaccgaagagtcactggtgaccttttgccgccgtcagctcacgggctacaaagtaccgaagctggtggagtttcgtgatgagttaccgaaatctaacgtcggaaaaattttgcgacgagaattacgtgacgaagcgcgcggcaaagtggacaataaagcctgataactctagaaataatttaaatggaattcgaagcttgggcccgaacaaaaactcatctcagaagaggatctgaatagcgccgtcgaccatcatcatcatcatcattgagtttaaacggtctccagcttggctgttttggcggatgagagaagattttcagcctgatacagattaaatcagaacgcagaagcggtctgataaaacagaatttgcctggcggcagtagcgcggtggtcccacctgaccccatgccgaactcagaagtgaaacgccgtagcgccgatggtagtgtggggtctccccatgcgagagtagggaactgccaggcatcaaataaaacgaaaggctcagtcgaaagactgggcctttcgttttatctgttgtttgtcggtgaacgctctcctgattaattaagacgtctaagaaaccattattatcatgacattaacctataaaaataggcgtatcacgaggccctttcgtcttcaagaattttataaaccgtggagcgggcaatactgagctgatgagcaatttccgttgcaccagtgcccttctgatgaagcgtcagcacgacgttcctgtccacggtacgcctgcggccaaatttgattcctttcagctttgcttcctgtcggccctcattcgtgcgctctaggatcctccggcgttcagcctgtgccacagccgacaggatggtgaccaccatttgccccatatcaccgtcggtactgatcccgtcgtcaataaaccgaaccgctacaccctgagcatcaaactcttttatcagttggatcatgtcggcggtgtcgcggccaagacggtcgagcttcttcaccagaatgacatcaccttcctccaccttcatcctcagcaaatccagcccttcccgatctgttgaactgccggatgccttgtcggtaaagatgcggttagcttttacccctgcatctttgagcgctgaggtctgcctcgtgaagaaggtgttgctgactcataccaggcctgaatcgccccatcatccagccagaaagtgagggagccacggttgatgagagctttgttgtaggtggaccagttggtgattttgaacttttgctttgccacggaacggtctgcgttgtcgggaagatgcgtgatctgatccttcaactcagcaaaagttcgatttattcaacaaagccgccgtcccgtcaagtcagcgtaatgccctaggaggcgcgccacggccgcgtcgaccccacgcccctctttaatacgacgggcaatttgcacttcagaaaatgaagagtttgctttagccataacaaaagtccagtatgctttttcacagcataactggactgatttcagtttacaactattctgtctagtttaagactttattgtcatagtttagatctattttgttcagtttaagactttattgtccgcccaca

SEQ ID NO: 18 - DNA, 20 bp, synthetic construct
  source 1..20: mol_type = other DNA; note = Synthetic primer
gatgctggtggcgaagctgt

SEQ ID NO: 19 - DNA, 23 bp, synthetic construct
  source 1..23: mol_type = other DNA; note = Synthetic primer
gttgcgacggtggtacgcataac

SEQ ID NO: 20 - DNA, 35 bp, synthetic construct
  source 1..35: mol_type = other DNA; note = Synthetic primer
gaggaataaaccatgcccattcttgaaagcgtggg

SEQ ID NO: 21 - DNA, 45 bp, synthetic construct
  source 1..45: mol_type = other DNA; note = Synthetic primer
agctggagaccgtttaaacttataaaccgctgtttgtcgcaaccg

SEQ ID NO: 22 - DNA, 663 bp, unidentified
  source 1..663: mol_type = genomic DNA; note = Uncultured bacterium RM44
atgcccattcttgaaagcgtgggtttcatgaagacgctatgggagagcggcggcgctcaggtcgccctgatggaatcgcgggaagagaccagccacatggtcggcatcctggaagggatcgccgccgaactctcgtggcgtcctggtacgcagcttcgcgattatcaggatagggcggcgcacctggccgttctggtcgggtcggagatcgtcggcggcttgcagatcgtcacgtcgccgtcagcggattgccttccctaccggctcgtctggccggaagtctgcgtgccggacggtgccgcaatcgcggacatcacgattctggcgctacggaaggaataccgcgcccgcttcaacctcttctggccgctgtgcgtcgagctctggcggcactgtgtcgcggagggtgccacggagatgcgcctggaggcaacgccggatacgctcaggctctaccgccgcatcggctggccgctggaggtcatcggcgacctgcgcctccactggaacgagccgtgcttcctgtgccggatggggatcgtagatgtcgcgggggcgatggttgtgcgggccttgcagtccgccacctatcaggcggtcctcgcggggatgagtcggcctgtggcgtcagcgtcgccggttgcgacaaacagcggtttatga